European Patent Application EP 4 282 421 A1, published November 29, 2023. Title: PROPHYLACTIC OR THERAPEUTIC AGENT FOR BENIGN ADULT FAMILIAL MYOCLONIC EPILEPSY. Applicant: RIKEN. The sequence listing filed with the application follows.

SEQUENCE LISTING (9 sequences)

SEQ ID NO: 1 - DNA, 20 bp, Homo sapiens
tgaaatgaaatgaaatgaaa

SEQ ID NO: 2 - DNA, 20 bp, Homo sapiens
tgaaatgaaataaaataaaa

SEQ ID NO: 3 - DNA, 20 bp, Homo sapiens
gtagttgacacttagtaggt

SEQ ID NO: 4 - DNA, 20 bp, Homo sapiens
aggataaggatagaaggctt

SEQ ID NO: 5 - DNA, 20 bp, Homo sapiens
gcaggaaaattgcttgaaac

SEQ ID NO: 6 - DNA, 20 bp, Homo sapiens
cacggtggctcatgcctgta

SEQ ID NO: 7 - DNA, 20 bp, Homo sapiens
taaaataaaataaaataaaa

SEQ ID NO: 8 - DNA, 21 bp, artificial
  Control Mixmer AntiSense Oligonucleotide
cacgcgagacacgcgagacga

SEQ ID NO: 9 - DNA, 20 bp, artificial
  Control Gapmer AntiSense Oligonucleotide
cctataggactatccaggaa